European Patent Application EP 4 703 382 A1, published March 4, 2026. Title: 一种抗PD-L1纳米抗体及其制备方法和应用. Applicant: 康立泰生物医药（青岛）有限公司. The sequence listing filed with the application follows.

SEQUENCE LISTING (48 sequences)

SEQ ID NO: 1 - protein, 10 aa, synthetic construct
GFTVSNSAVS

SEQ ID NO: 2 - protein, 9 aa, synthetic construct
LIDSNRNTV

SEQ ID NO: 3 - protein, 8 aa, synthetic construct
KGIWGSTL

SEQ ID NO: 4 - protein, 10 aa, synthetic construct
GSIFRITPVA

SEQ ID NO: 5 - protein, 9 aa, synthetic construct
VITDNGSTD

SEQ ID NO: 6 - protein, 9 aa, synthetic construct
SRARPVRWT

SEQ ID NO: 7 - protein, 10 aa, synthetic construct
GFTFSTSFVS

SEQ ID NO: 8 - protein, 10 aa, synthetic construct
RISPGGASTS

SEQ ID NO: 9 - protein, 13 aa, synthetic construct
REIYSGRFSGFDY

SEQ ID NO: 10 - protein, 10 aa, synthetic construct
GIISDINMVA

SEQ ID NO: 11 - protein, 9 aa, synthetic construct
KIFRGGSTY

SEQ ID NO: 12 - protein, 14 aa, synthetic construct
ARIQIRADRDYSDY

SEQ ID NO: 13 - protein, 115 aa, synthetic construct
QVQLQESGGGLVQPGGSLTLSCAASGFTVSNSAVSWARQAPGKGLEWVSLIDSNRNTVYAQSVRGRFTISRDNVKNTVYLQMNSLKPEDTAVYYCAKGIWGSTLTGQGTQVTVSS

SEQ ID NO: 14 - protein, 116 aa, synthetic construct
QVQLQESGGGLVQPGGSLRLSCAGSGSIFRITPVAWYRQAPEKQRELVAVITDNGSTDYGDFVKGRFTISRDNAKNTVYLQMNSLKPEDTAVYYCNSRARPVRWTWGQGTQVTVSS

SEQ ID NO: 15 - protein, 121 aa, synthetic construct
QVQLQESGGGLVQPGGSLRLSCAASGFTFSTSFVSWVRQAPGKGLEWVSRISPGGASTSYADSVKGRFTISRDNAENTLYLQMNSLKPEDTALYYCAREIYSGRFSGFDYWGQGTQVTVSS

SEQ ID NO: 16 - protein, 121 aa, synthetic construct
QVQLQESGGGLVQPGGSLRLSCAASGIISDINMVAWYRQAPGKQRELVAKIFRGGSTYYTDFVKGRFTISRENAKNTVYLQMNSLKPDDTAVYYCNARIQIRADRDYSDYWGQGTQVTVSS

SEQ ID NO: 17 - protein, 238 aa, synthetic construct
MRIFAVFIFMTYWHLLNAFTVTVPKDLYVVEYGSNMTIECKFPVEKQLDLAALIVYWEMEDKNIIQFVHGEEDLKVQHSSYRQRARLLKDQLSLGNAALQITDVKLQDAGVYRCMISYGGADYKRITVKVNAPYNKINQRILVVDPVTSEHELTCQAEGYPKAEVIWTSSDHQVLSGKTTTTNSKREEKLFNVTSTLRINTTTNEIFYCTFRRLDPEENHTAELVIPELPLAHPPNER

SEQ ID NO: 18 - protein, 244 aa, synthetic construct
MRIFAVFIFMTYWHLLNAFTVTVPKDLYVVEYGSNMTIECKFPVEKQLDLAALIVYWEMEDKNIIQFVHGEEDLKVQHSSYRQRARLLKDQLSLGNAALQITDVKLQDAGVYRCMISYGGADYKRITVKVNAPYNKINQRILVVDPVTSEHELTCQAEGYPKAEVIWTSSDHQVLSGKTTTTNSKREEKLFNVTSTLRINTTTNEIFYCTFRRLDPEENHTAELVIPELPLAHPPNERHHHHHH

SEQ ID NO: 19 - protein, 470 aa, synthetic construct
MRIFAVFIFMTYWHLLNAFTVTVPKDLYVVEYGSNMTIECKFPVEKQLDLAALIVYWEMEDKNIIQFVHGEEDLKVQHSSYRQRARLLKDQLSLGNAALQITDVKLQDAGVYRCMISYGGADYKRITVKVNAPYNKINQRILVVDPVTSEHELTCQAEGYPKAEVIWTSSDHQVLSGKTTTTNSKREEKLFNVTSTLRINTTTNEIFYCTFRRLDPEENHTAELVIPELPLAHPPNEREPKSCDKTHTCPPCPAPELLGGPSVFLFPPKPKDTLMISRTPEVTCVVVDVSHEDPEVKFNWYVDGVEVHNAKTKPREEQYNSTYRVVSVLTVLHQDWLNGKEYKCKVSNKALPAPIEKTISKAKGQPREPQVYTLPPSRDELTKNQVSLTCLVKGFYPSDIAVEWESNGQPENNYKTTPPVLDSDGSFFLYSKLTVDKSRWQQGNVFSCSVMHEALHNHYTQKSLSLSPGK

SEQ ID NO: 20 - protein, 374 aa, synthetic construct
PGWFLDSPDRPWNPPTFSPALLVVTEGDNATFTCSFSNTSESFVLNWYRMSPSNQTDKLAAFPEDRSQPGQDCRFRVTQLPNGRDFHMSVVRARRNDSGTYLCGAISLAPKAQIKESLRAELRVTERRAEVPTAHPSPSPRPAGQFQDKTHTCPPCPAPELLGGPSVFLFPPKPKDTLMISRTPEVTCVVVDVSHEDPEVKFNWYVDGVEVHNAKTKPREEQYNSTYRVVSVLTVLHQDWLNGKEYKCKVSNKALPAPIEKTISKAKGQPREPQVYTLPPSRDELTKNQVSLTCLVKGFYPSDIAVEWESNGQPENNYKTTPPVLDSDGSFFLYSKLTVDKSRWQQGNVFSCSVMHEALHNHYTQKSLSLSPGK

SEQ ID NO: 21 - protein, 232 aa, synthetic construct
EPKSCDKTHTCPPCPAPELLGGPSVFLFPPKPKDTLMISRTPEVTCVVVDVSHEDPEVKFNWYVDGVEVHNAKTKPREEQYNSTYRVVSVLTVLHQDWLNGKEYKCKVSNKALPAPIEKTISKAKGQPREPQVYTLPPSRDELTKNQVSLTCLVKGFYPSDIAVEWESNGQPENNYKTTPPVLDSDGSFFLYSKLTVDKSRWQQGNVFSCSVMHEALHNHYTQKSLSLSPGK

SEQ ID NO: 22 - protein, 360 aa, synthetic construct
QVQLVESGGGLVQPGGSLRLSCAASGKMSSRRCMAWFRQAPGKERERVAKLLTTSGSTYLADSVKGRFTISRDNSKNTVYLQMNSLRAEDTAVYYCAADSFEDPTCTLVTSSGAFQYWGQGTLVTVSSEPKSSDKTHTCPPCPAPELLGGPSVFLFPPKPKDTLMISRTPEVTCVVVAVSHEDPEVKFNWYVDGVEVHNAKTKPREEQYNSTYRVVSVLTVLHQDWLNGKEYKCKVSNKALPAGIEKTISKAKGQPREPQVYTLPPSRDELTKNQVSLTCLVKGFYPSDIAVEWESNGQPENNYKTTPPVLDSDGSFFLYSKLTVDKSRWQQGNVFSCSVMHEALHNHYTQKSLSLSPGK

SEQ ID NO: 23 - protein, 115 aa, synthetic construct
EVQLLESGGGLVQPGGSLRLSCAASGFTVSNSAVSWARQAPGKGLEWVSLIDSNRNTVYAQSVRGRFTISRDNSKNTVYLQMNSLRAEDTAVYYCAKGIWGSTLWGQGTTVTVSS

SEQ ID NO: 24 - protein, 115 aa, synthetic construct
QVQLVESGGGLVKPGGSLRLSCAASGFTVSNSAVSWARQAPGKGLEWVSLIDSNRNTVYAQSVRGRFTISRDNAKNSVYLQMNSLRAEDTAVYYCAKGIWGSTLWGQGTTVTVSS

SEQ ID NO: 25 - protein, 115 aa, synthetic construct
QVQLLESGGGLVQPGGSLRLSCAASGFTVSNSAVSWARQAPGKGLEWVSLIDSNRNTVYAQSVRGRFTISRDNSKNTVYLQMNSLRAEDTAVYYCAKGIWGSTLWGQGTTVTVSS

SEQ ID NO: 26 - protein, 115 aa, synthetic construct
EVQLQESGGGLVQPGGSLRLSCAASGFTVSNSAVSWARQAPGKGLEWVSLIDSNRNTVYAQSVRGRFTISRDNSKNTVYLQMNSLRAEDTAVYYCAKGIWGSTLWGQGTTVTVSS

SEQ ID NO: 27 - protein, 114 aa, synthetic construct
EVQLLESGGGLVQPGGSLRLSCAASGFTVSNSAVSWARQAPGKGLEWVSLIDSNRNTVYAQSVRGRFTISRDNVKNTVYLQMNSLRAEDTAVYYCAKGWGSTLWGQGTTVTVSS

SEQ ID NO: 28 - protein, 115 aa, synthetic construct
EVQLLESGGGLVQPGGSLRLSCAASGFTVSNSAVSWARQAPGKGLEWVSLIDSNRNTVYAQSVRGRFTISRDNSKNTVYLQMNSLKAEDTAVYYCAKGIWGSTLWGQGTTVTVSS

SEQ ID NO: 29 - protein, 115 aa, synthetic construct
EVQLLESGGGLVQPGGSLRLSCAASGFTVSNSAVSWARQAPGKGLEWVSLIDSNRNTVYAQSVRGRFTISRDNSKNTVYLQMNSLRPEDTAVYYCAKGIWGSTLWGQGTTVTVSS

SEQ ID NO: 30 - protein, 115 aa, synthetic construct
EVQLLESGGGLVQPGGSLRLSCAASGFTVSNSAVSWARQAPGKGLEWVSLIDSNRNTVYAQSVRGRFTISRDNSKNTVYLQMNSLRAEDTAVYYCAKGIWGSTLTGQGTTVTVSS

SEQ ID NO: 31 - protein, 115 aa, synthetic construct
EVQLLESGGGLVQPGGSLRLSCAASGFTVSNSAVSWARQAPGKGLEWVSLIDSNRNTVYAQSVRGRFTISRDNSKNTVYLQMNSLRAEDTAVYYCAKGIWGSTLWGQGTQVTVSS

SEQ ID NO: 32 - protein, 115 aa, synthetic construct
EVQLLESGGGLVQPGGSLRLSCAASGFTVSNSAVSWARQAPGKGLEWVSLIASNRNTVYAQSVRGRFTISRDNSKNTVYLQMNSLRAEDTAVYYCAKGIWGSTLWGQGTTVTVSS

SEQ ID NO: 33 - protein, 115 aa, synthetic construct
QVQLQESGGGLVKPGGSLRLSCAASGFTVSNSAVSWARQAPGKGLEWVSLIDSNRNTVYAQSVRGRFTISRDNAKNSVYLQMNSLRAEDTAVYYCAKGIWGSTLWGQGTTVTVSS

SEQ ID NO: 34 - protein, 115 aa, synthetic construct
QVQLVESGGGLVQPGGSLRLSCAASGFTVSNSAVSWARQAPGKGLEWVSLIDSNRNTVYAQSVRGRFTISRDNAKNSVYLQMNSLRAEDTAVYYCAKGIWGSTLWGQGTTVTVSS

SEQ ID NO: 35 - protein, 115 aa, synthetic construct
QVQLVESGGGLVKPGGSLTLSCAASGFTVSNSAVSWARQAPGKGLEWVSLIDSNRNTVYAQSVRGRFTISRDNAKNSVYLQMNSLRAEDTAVYYCAKGIWGSTLWGQGTTVTVSS

SEQ ID NO: 36 - protein, 115 aa, synthetic construct
QVQLVESGGGLVKPGGSLRLSCAASGFTVSNSAVSWARQAPGKGLEWVSLIDSNRNTVYAQSVRGRFTISRDNVKNSVYLQMNSLRAEDTAVYYCAKGIWGSTLWGQGTTVTVSS

SEQ ID NO: 37 - protein, 115 aa, synthetic construct
QVQLVESGGGLVKPGGSLRLSCAASGFTVSNSAVSWARQAPGKGLEWVSLIDSNRNTVYAQSVRGRFTISRDNAKNTVYLQMNSLRAEDTAVYYCAKGIWGSTLWGQGTTVTVSS

SEQ ID NO: 38 - protein, 115 aa, synthetic construct
QVQLVESGGGLVKPGGSLRLSCAASGFTVSNSAVSWARQAPGKGLEWVSLIDSNRNTVYAQSVRGRFTISRDNAKNSVYLQMNSLKAEDTAVYYCAKGIWGSTLWGQGTTVTVSS

SEQ ID NO: 39 - protein, 115 aa, synthetic construct
QVQLVESGGGLVKPGGSLRLSCAASGFTVSNSAVSWARQAPGKGLEWVSLIDSNRNTVYAQSVRGRFTISRDNAKNSVYLQMNSLRPEDTAVYYCAKGIWGSTLWGQGTTVTVSS

SEQ ID NO: 40 - protein, 115 aa, synthetic construct
QVQLVESGGGLVKPGGSLRLSCAASGFTVSNSAVSWARQAPGKGLEWVSLIDSNRNTVYAQSVRGRFTISRDNAKNSVYLQMNSLRAEDTAVYYCAKGIWGSTLTGQGTTVTVSS

SEQ ID NO: 41 - protein, 115 aa, synthetic construct
QVQLVESGGGLVKPGGSLRLSCAASGFTVSNSAVSWARQAPGKGLEWVSLIDSNRNTVYAQSVRGRFTISRDNAKNSVYLQMNSLRAEDTAVYYCAKGIWGSTLWGQGTQVTVSS

SEQ ID NO: 42 - protein, 115 aa, synthetic construct
QVQLVESGGGLVKPGGSLRLSCAASGFTVSNSAVSWARQAPGKGLEWVSLIASNRNTVYAQSVRGRFTISRDNAKNSVYLQMNSLRAEDTAVYYCAKGIWGSTLWGQGTTVTVSS

SEQ ID NO: 43 - DNA, 23 bp, synthetic construct
  source 1..23: mol_type = other DNA
gtcctggctgctcttctacaagg

SEQ ID NO: 44 - DNA, 23 bp, synthetic construct
  source 1..23: mol_type = other DNA
ggtacgtgctgttgaactgttcc

SEQ ID NO: 45 - DNA, 35 bp, synthetic construct
  source 1..35: mol_type = other DNA
atggcccaggtgcagctgcaggagtctggrggagg

SEQ ID NO: 46 - DNA, 27 bp, synthetic construct
  source 1..27: mol_type = other DNA
gtggtgtgaggagacggtgacctgggt

SEQ ID NO: 47 - DNA, 39 bp, synthetic construct
  source 1..39: mol_type = other DNA
ccttaagggcgtgcagtgccaggtgcagctgcaggagtc

SEQ ID NO: 48 - DNA, 37 bp, synthetic construct
  source 1..37: mol_type = other DNA
gatttgggctcgctagctgaggagacggtgacctggg